European Patent Application EP 4 123 029 A1, published January 25, 2023. Title: In vitro Transcript mRNA and Pharmaceutical Composition Containing Thereof. Applicant: abion SNU R&DB FOUNDATION. The sequence listing filed with the application follows.

SEQUENCE LISTING (5 sequences)

SEQ ID NO: 1 - DNA, 1431 bp, Artificial Sequence
  Tomato fluorecent proein gene
atggtgagcaagggcgaggaggtcatcaaagagttcatgcgcttcaaggtgcgcatggagggctccatgaacggccacgagttcgagatcgagggcgagggcgagggccgcccctacgagggcacccagaccgccaagctgaaggtgaccaagggcggccccctgcccttcgcctgggacatcctgtccccccagttcatgtacggctccaaggcgtacgtgaagcaccccgccgacatccccgattacaagaagctgtccttccccgagggcttcaagtgggagcgcgtgatgaacttcgaggacggcggtctggtgaccgtgacccaggactcctccctgcaggacggcacgctgatctacaaggtgaagatgcgcggcaccaacttcccccccgacggccccgtaatgcagaagaagaccatgggctgggaggcctccaccgagcgcctgtacccccgcgacggcgtgctgaagggcgagatccaccaggccctgaagctgaaggacggcggccactacctggtggagttcaagaccatctacatggccaagaagcccgtgcaactgcccggctactactacgtggacaccaagctggacatcacctcccacaacgaggactacaccatcgtggaacagtacgagcgctccgagggccgccaccacctgttcctggggcatggcaccggcagcaccggcagcggcagctccggcaccgcctcctccgaggacaacaacatggccgtcatcaaagagttcatgcgcttcaaggtgcgcatggagggctccatgaacggccacgagttcgagatcgagggcgagggcgagggccgcccctacgagggcacccagaccgccaagctgaaggtgaccaagggcggccccctgcccttcgcctgggacatcctgtccccccagttcatgtacggctccaaggcgtacgtgaagcaccccgccgacatccccgattacaagaagctgtccttccccgagggcttcaagtgggagcgcgtgatgaacttcgaggacggcggtctggtgaccgtgacccaggactcctccctgcaggacggcacgctgatctacaaggtgaagatgcgcggcaccaacttcccccccgacggccccgtaatgcagaagaagaccatgggctgggaggcctccaccgagcgcctgtacccccgcgacggcgtgctgaagggcgagatccaccaggccctgaagctgaaggacggcggccactacctggtggagttcaagaccatctacatggccaagaagcccgtgcaactgcccggctactactacgtggacaccaagctggacatcacctcccacaacgaggactacaccatcgtggaacagtacgagcgctccgagggccgccaccacctgttcctgtacggcatggacgagctgtacaagtaa

SEQ ID NO: 2 - DNA, 1610 bp, Artificial Sequence
  in vitro transcription template pDNA
ggttccgcgcacatttccccgaaaagtgccacctgacgtctaagaaaccattattatcatgacattaacctataaaaataggcgtatcacgaggccctttcgtctcgcgcgtttcggtgatgacggtgaaaacctctgacacatgcagctcccggagacggtcacagcttgtctgtaagcggatgccgggagcagacaagcccgtcagggcgcgtcagcgggtgttggcgggtgtcggggctggcttaactatgcggcatcagagcagattgtactgagagtgcaccatatgcggtgtgaaataccgcacagatgcgtaaggagaaaataccgcatcaggcgccattcgccattcaggctgcgcaactgttgggaagggcgatcggtgcgggcctcttcgctattacgccagctggcgaaagggggatgtgctgcaaggcgattaagttgggtaacgccagggttttcccagtcacgacgttgtaaaacgacggccagtgaattgtaatacgactcactatagggcgaattaattcgagctcggtacccagcttgcttgttctttttgcagaagctcagaataaacgctcaactttggcagatcaattccccatcatcgatgaattcgccaccatgaaattcagctgggtcatgttcttcctgatggcagtggttacaggggtcaattcagagaagatcaagctgaatgccaagatgaatatcctgatccgggacaagagattccactacgataggaacaacatcgccgtgggcgccgacgagagcgtggtgaaggaggcccacagagaagtgattaactcttctaccgagggactgctgctgaacattgacaaggacatccggaagatcctgagcggctatatcgtggagatcgaggataccgagggcctgaaagaagtgatcaatgacagatacgacatgctgaacatcagcagcctgcggcaggatggcaagacctttatcgacttcaaaaaatacaatgataagctgccactgtacatcagcaaccccaactataaggtgaacgtgtacgccgtgacaaaggagaataccatcatcaatccttccgagaacggcgataccagcaccaatggcattaagaagattctgattttcagcaaaaagggatacgaaatcggctgaaagcttgatctggttaccactaaaccagcctcaagaacacccgaatggagtctctaagctacataataccaacttacactttacaaaatgttgtcccccaaaatgtagccattcgtatctgctcctaataaaaagaaagtttcttcacattctaaaaaaaaataaaaaaaaataaaaaaaaataaaaaaaaataaaaaaaaataaaaaaaaataaaaaaaaataaaaaaaaataaaaaaaaataaaaaaaaataaaaaaaaataaaaaaaaaacgaagagctagcttaagtattctatagtgtcgcttcctcgctcactgactcgctgcgctcggtcgttcggctgcggcgagcggtatcagctcactcaaaggcggtaatacggttatccacagaatcaggggataacgcaggaaagaacatgtgagcaaaaggccagcaaaagg

SEQ ID NO: 3 - DNA, 34 bp, Artificial Sequence
  primer
atgaattcgccaccatggtgagcaagggcgagga

SEQ ID NO: 4 - DNA, 28 bp, Artificial Sequence
  primer
ataagcttttacttgtacagctcgtcca

SEQ ID NO: 5 - RNA, 1815 nt, Artificial Sequence
  in vitro transcripti of Tomato fluorecent protein gene
gggcgaauuaauucgagcucgguacccagcuugcuuguucuuuuugcagaagcucagaauaaacgcucaacuuuggcagaucaauuccccaucaucgaugaauucgccaccauggugagcaagggcgaggaggucaucaaagaguucaugcgcuucaaggugcgcauggagggcuccaugaacggccacgaguucgagaucgagggcgagggcgagggccgccccuacgagggcacccagaccgccaagcugaaggugaccaagggcggcccccugcccuucgccugggacauccuguccccccaguucauguacggcuccaaggcguacgugaagcaccccgccgacauccccgauuacaagaagcuguccuuccccgagggcuucaagugggagcgcgugaugaacuucgaggacggcggucuggugaccgugacccaggacuccucccugcaggacggcacgcugaucuacaaggugaagaugcgcggcaccaacuucccccccgacggccccguaaugcagaagaagaccaugggcugggaggccuccaccgagcgccuguacccccgcgacggcgugcugaagggcgagauccaccaggcccugaagcugaaggacggcggccacuaccugguggaguucaagaccaucuacauggccaagaagcccgugcaacugcccggcuacuacuacguggacaccaagcuggacaucaccucccacaacgaggacuacaccaucguggaacaguacgagcgcuccgagggccgccaccaccuguuccuggggcauggcaccggcagcaccggcagcggcagcuccggcaccgccuccuccgaggacaacaacauggccgucaucaaagaguucaugcgcuucaaggugcgcauggagggcuccaugaacggccacgaguucgagaucgagggcgagggcgagggccgccccuacgagggcacccagaccgccaagcugaaggugaccaagggcggcccccugcccuucgccugggacauccuguccccccaguucauguacggcuccaaggcguacgugaagcaccccgccgacauccccgauuacaagaagcuguccuuccccgagggcuucaagugggagcgcgugaugaacuucgaggacggcggucuggugaccgugacccaggacuccucccugcaggacggcacgcugaucuacaaggugaagaugcgcggcaccaacuucccccccgacggccccguaaugcagaagaagaccaugggcugggaggccuccaccgagcgccuguacccccgcgacggcgugcugaagggcgagauccaccaggcccugaagcugaaggacggcggccacuaccugguggaguucaagaccaucuacauggccaagaagcccgugcaacugcccggcuacuacuacguggacaccaagcuggacaucaccucccacaacgaggacuacaccaucguggaacaguacgagcgcuccgagggccgccaccaccuguuccuguacggcauggacgagcuguacaaguaaaagcuugaucugguuaccacuaaaccagccucaagaacacccgaauggagucucuaagcuacauaauaccaacuuacacuuuacaaaauguugucccccaaaauguagccauucguaucugcuccuaauaaaaagaaaguuucuucacauucuaaaaaaaaauaaaaaaaaauaaaaaaaaauaaaaaaaaauaaaaaaaaauaaaaaaaaauaaaaaaaaauaaaaaaaaauaaaaaaaaauaaaaaaaaauaaaaaaaaauaaaaaaaaaa